European Patent Application EP 4 553 085 A1, published May 14, 2025. Title: Isolated antigen-binding protein and use thereof. Applicant: 杭州尚健生物技术有限公司. The sequence listing filed with the application follows.

SEQUENCE LISTING (92 sequences)

SEQ ID NO: 1 - protein, 5 aa, synthetic construct
  REGION 1..5: note = 1A2-7/3A2-18/RB4-G1-018/RB4-G1-019/RB4-G1-020/RB4-G1-022/3G9-1 HCDR1
SYWMH

SEQ ID NO: 2 - protein, 17 aa, synthetic construct
  REGION 1..17: note = 1A2-7/3A2-18/RB4-G1-018/RB4-G1-019/RB4-G1-020/RB4-G1-022/3G9-1 HCDR2
EINPSNGRTNYNEKFKS

SEQ ID NO: 3 - protein, 11 aa, synthetic construct
  REGION 1..11: note = 1A2-7/3A2-18/RB4-G1-018/RB4-G1-019/RB4-G1-020/RB4-G1-022 HCDR3
DRYDEGNAMDY

SEQ ID NO: 4 - protein, 30 aa, synthetic construct
  REGION 1..30: note = 1A2-7/3G9-1 H-FR1
QVQLQQPGAELVKPGASVKLSCKASGYTFT

SEQ ID NO: 5 - protein, 14 aa, synthetic construct
  REGION 1..14: note = 1A2-7/3A2-18/3G9-1 H-FR2
WVKQRPGQGLEWIG

SEQ ID NO: 6 - protein, 32 aa, synthetic construct
  REGION 1..32: note = 1A2-7 H-FR3
KATLTVDKSSSTAYMQLNSLTSEDSAVYYCAR

SEQ ID NO: 7 - protein, 11 aa, synthetic construct
  REGION 1..11: note = 1A2-7/3A2-18/3G9-1/5E11-2 H-FR4
WGQGTSVTVSS

SEQ ID NO: 8 - protein, 120 aa, synthetic construct
  REGION 1..120: note = 1A2-7 VH
QVQLQQPGAELVKPGASVKLSCKASGYTFTSYWMHWVKQRPGQGLEWIGEINPSNGRTNYNEKFKSKATLTVDKSSSTAYMQLNSLTSEDSAVYYCARDRYDEGNAMDYWGQGTSVTVSS

SEQ ID NO: 9 - protein, 11 aa, synthetic construct
  REGION 1..11: note = 1A2-7/3A2-18/RB4-G1-018/RB4-G1-019/RB4-G1-020/RB4-G1-022 LCDR1
RASQDITNYLN

SEQ ID NO: 10 - protein, 7 aa, synthetic construct
  REGION 1..7: note = 1A2-7/3A2-18/RB4-G1-018/RB4-G1-019/RB4-G1-020/RB4-G1-022/3G9-1 LCDR2
YTSRLHS

SEQ ID NO: 11 - protein, 9 aa, synthetic construct
  REGION 1..9: note = 1A2-7/3A2-18/RB4-G1-018/RB4-G1-019/RB4-G1-020/RB4-G1-022 LCDR3
QQGDTLPRT

SEQ ID NO: 12 - protein, 23 aa, synthetic construct
  REGION 1..23: note = 1A2-7/3A2-18 L-FR1
DIVMTQTTSSLSASLGDRVTISC

SEQ ID NO: 13 - protein, 15 aa, synthetic construct
  REGION 1..15: note = 1A2-7/3A2-18/3G9-1 L-FR2
WYQQKPDGTVKLLIY

SEQ ID NO: 14 - protein, 32 aa, synthetic construct
  REGION 1..32: note = 1A2-7/3A2-18/3G9-1 L-FR3
GVPSRFSGSGSGTDYSLTISNLEQEDIATYFC

SEQ ID NO: 15 - protein, 10 aa, synthetic construct
  REGION 1..10: note = 1A2-7/3A2-18/3G9-1/5E11-2 L-FR4
FGGGTKLEIK

SEQ ID NO: 16 - protein, 107 aa, synthetic construct
  REGION 1..107: note = 1A2-7/3A2-18 VL
DIVMTQTTSSLSASLGDRVTISCRASQDITNYLNWYQQKPDGTVKLLIYYTSRLHSGVPSRFSGSGSGTDYSLTISNLEQEDIATYFCQQGDTLPRTFGGGTKLEIK

SEQ ID NO: 17 - protein, 30 aa, synthetic construct
  REGION 1..30: note = 3A2-18 H-FR1
EVQLQQPGAELVKPGASVKLSCKASGYTFT

SEQ ID NO: 18 - protein, 32 aa, synthetic construct
  REGION 1..32: note = 3A2-18 H-FR3
KATLTVDKSSSTAYVQLNSLTSEDSAVYYCAR

SEQ ID NO: 19 - protein, 120 aa, synthetic construct
  REGION 1..120: note = 3A2-18 VH
EVQLQQPGAELVKPGASVKLSCKASGYTFTSYWMHWVKQRPGQGLEWIGEINPSNGRTNYNEKFKSKATLTVDKSSSTAYVQLNSLTSEDSAVYYCARDRYDEGNAMDYWGQGTSVTVSS

SEQ ID NO: 20 - protein, 12 aa, synthetic construct
  REGION 1..12: note = 3G9-1 HCDR3
GIYYGYDYAMDY

SEQ ID NO: 21 - protein, 32 aa, synthetic construct
  REGION 1..32: note = 3G9-1 H-FR3
KATLIVDKSSSTAYMQLSSLTSEDSAVYYCAR

SEQ ID NO: 22 - protein, 121 aa, synthetic construct
  REGION 1..121: note = 3G9-1 VH
QVQLQQPGAELVKPGASVKLSCKASGYTFTSYWMHWVKQRPGQGLEWIGEINPSNGRTNYNEKFKSKATLIVDKSSSTAYMQLSSLTSEDSAVYYCARGIYYGYDYAMDYWGQGTSVTVSS

SEQ ID NO: 23 - protein, 11 aa, synthetic construct
  REGION 1..11: note = 3G9-1 LCDR1
RASQDISNYLN

SEQ ID NO: 24 - protein, 9 aa, synthetic construct
  REGION 1..9: note = 3G9-1 LCDR3
QQGNTLPPT

SEQ ID NO: 25 - protein, 23 aa, synthetic construct
  REGION 1..23: note = 3G9-1 L-FR1
DIQMTHTTSSLSASLGDRVTISC

SEQ ID NO: 26 - protein, 107 aa, synthetic construct
  REGION 1..107: note = 3G9-1 VL
DIQMTHTTSSLSASLGDRVTISCRASQDISNYLNWYQQKPDGTVKLLIYYTSRLHSGVPSRFSGSGSGTDYSLTISNLEQEDIATYFCQQGNTLPPTFGGGTKLEIK

SEQ ID NO: 27 - protein, 5 aa, synthetic construct
  REGION 1..5: note = 5E11-2 HCDR1
DAWMD

SEQ ID NO: 28 - protein, 19 aa, synthetic construct
  REGION 1..19: note = 5E11-2 HCDR2
EIRSKPNNHATYYAESVKG

SEQ ID NO: 29 - protein, 8 aa, synthetic construct
  REGION 1..8: note = 5E11-2 HCDR3
TTDYSMDY

SEQ ID NO: 30 - protein, 30 aa, synthetic construct
  REGION 1..30: note = 5E11-2 H-FR1
EVKLEESGGGLVQPGGSMKLSCAASGFTFS

SEQ ID NO: 31 - protein, 14 aa, synthetic construct
  REGION 1..14: note = 5E11-2 H-FR2
WVRQSPEKGLEWVA

SEQ ID NO: 32 - protein, 32 aa, synthetic construct
  REGION 1..32: note = 5E11-2 H-FR3
RFTISRDDSKSSVYLQMNSLRAEDTGIYYCTR

SEQ ID NO: 33 - protein, 119 aa, synthetic construct
  REGION 1..119: note = 5E11-2 VH
EVKLEESGGGLVQPGGSMKLSCAASGFTFSDAWMDWVRQSPEKGLEWVAEIRSKPNNHATYYAESVKGRFTISRDDSKSSVYLQMNSLRAEDTGIYYCTRTTDYSMDYWGQGTSVTVSS

SEQ ID NO: 34 - protein, 15 aa, synthetic construct
  REGION 1..15: note = 5E11-2 LCDR1
RASQSVSASSYSYMH

SEQ ID NO: 35 - protein, 7 aa, synthetic construct
  REGION 1..7: note = 5E11-2 LCDR2
YASNLQS

SEQ ID NO: 36 - protein, 9 aa, synthetic construct
  REGION 1..9: note = 5E11-2 LCDR3
QHSWEIPRT

SEQ ID NO: 37 - protein, 23 aa, synthetic construct
  REGION 1..23: note = 5E11-2 L-FR1
DIQMTQSPASLAVSLGQRATISC

SEQ ID NO: 38 - protein, 15 aa, synthetic construct
  REGION 1..15: note = 5E11-2 L-FR2
WYQQKPGQPPKLLIK

SEQ ID NO: 39 - protein, 32 aa, synthetic construct
  REGION 1..32: note = 5E11-2 L-FR3
GVPARFSGSGSGTDFTLNIHPVEEEDSATYYC

SEQ ID NO: 40 - protein, 111 aa, synthetic construct
  REGION 1..111: note = 5E11-2 VL
DIQMTQSPASLAVSLGQRATISCRASQSVSASSYSYMHWYQQKPGQPPKLLIKYASNLQSGVPARFSGSGSGTDFTLNIHPVEEEDSATYYCQHSWEIPRTFGGGTKLEIK

SEQ ID NO: 41 - protein, 30 aa, synthetic construct
  REGION 1..30: note = RB4-G1-018/RB4-G1-019/RB4-G1-020/RB4-G1-022 H-FR1
QVQLVQSGAEVKKPGASVKVSCKASGYTFT

SEQ ID NO: 42 - protein, 14 aa, synthetic construct
  REGION 1..14: note = RB4-G1-018/RB4-G1-022 H-FR2
WVRQAPGQGLEWIG

SEQ ID NO: 43 - protein, 32 aa, synthetic construct
  REGION 1..32: note = RB4-G1-018/RB4-G1-022 H-FR3
RATLTVDKSTSTAYMELSSLRSEDTAVYYCAR

SEQ ID NO: 44 - protein, 11 aa, synthetic construct
  REGION 1..11: note = RB4-G1-018/RB4-G1-019/RB4-G1-020/RB4-G1-022 H-FR4
WGQGTTVTVSS

SEQ ID NO: 45 - protein, 120 aa, synthetic construct
  REGION 1..120: note = RB4-G1-018/RB4-G1-022 VH
QVQLVQSGAEVKKPGASVKVSCKASGYTFTSYWMHWVRQAPGQGLEWIGEINPSNGRTNYNEKFKSRATLTVDKSTSTAYMELSSLRSEDTAVYYCARDRYDEGNAMDYWGQGTTVTVSS

SEQ ID NO: 46 - protein, 450 aa, synthetic construct
  REGION 1..450: note = RB4-G1-018/RB4-G1-022 heavy chain
QVQLVQSGAEVKKPGASVKVSCKASGYTFTSYWMHWVRQAPGQGLEWIGEINPSNGRTNYNEKFKSRATLTVDKSTSTAYMELSSLRSEDTAVYYCARDRYDEGNAMDYWGQGTTVTVSSASTKGPSVFPLAPSSKSTSGGTAALGCLVKDYFPEPVTVSWNSGALTSGVHTFPAVLQSSGLYSLSSVVTVPSSSLGTQTYICNVNHKPSNTKVDKKVEPKSCDKTHTCPPCPAPELLGGPSVFLFPPKPKDTLMISRTPEVTCVVVDVSHEDPEVKFNWYVDGVEVHNAKTKPREEQYNSTYRVVSVLTVLHQDWLNGKEYKCKVSNKALPAPIEKTISKAKGQPREPQVYTLPPSRDELTKNQVSLTCLVKGFYPSDIAVEWESNGQPENNYKTTPPVLDSDGSFFLYSKLTVDKSRWQQGNVFSCSVMHEALHNHYTQKSLSLSPGK

SEQ ID NO: 47 - protein, 23 aa, synthetic construct
  REGION 1..23: note = RB4-G1-018/RB4-G1-019/RB4-G1-020/RB4-G1-022 L-FR1
DIQMTQSPSSLSASVGDRVTITC

SEQ ID NO: 48 - protein, 15 aa, synthetic construct
  REGION 1..15: note = RB4-G1-018/RB4-G1-019/RB4-G1-020/RB4-G1-022 L-FR2
WYQQKPGKAPKLLIY

SEQ ID NO: 49 - protein, 32 aa, synthetic construct
  REGION 1..32: note = RB4-G1-018/RB4-G1-019/RB4-G1-020 L-FR3
GVPSRFSGSGSGTEYTLTISSLQPDDFATYYC

SEQ ID NO: 50 - protein, 10 aa, synthetic construct
  REGION 1..10: note = RB4-G1-018/RB4-G1-019/RB4-G1-020/RB4-G1-022 L-FR4
FGQGTRLEIK

SEQ ID NO: 51 - protein, 107 aa, synthetic construct
  REGION 1..107: note = RB4-G1-018/RB4-G1-019/RB4-G1-020 VL
DIQMTQSPSSLSASVGDRVTITCRASQDITNYLNWYQQKPGKAPKLLIYYTSRLHSGVPSRFSGSGSGTEYTLTISSLQPDDFATYYCQQGDTLPRTFGQGTRLEIK

SEQ ID NO: 52 - protein, 214 aa, synthetic construct
  REGION 1..214: note = RB4-G1-018/RB4-G1-019/RB4-G1-020 light chain
DIQMTQSPSSLSASVGDRVTITCRASQDITNYLNWYQQKPGKAPKLLIYYTSRLHSGVPSRFSGSGSGTEYTLTISSLQPDDFATYYCQQGDTLPRTFGQGTRLEIKRTVAAPSVFIFPPSDEQLKSGTASVVCLLNNFYPREAKVQWKVDNALQSGNSQESVTEQDSKDSTYSLSSTLTLSKADYEKHKVYACEVTHQGLSSPVTKSFNRGEC

SEQ ID NO: 53 - protein, 14 aa, synthetic construct
  REGION 1..14: note = RB4-G1-019/RB4-G1-020 H-FR2
WVRQAPGQGLEWMG

SEQ ID NO: 54 - protein, 32 aa, synthetic construct
  REGION 1..32: note = RB4-G1-019 H-FR3
RVTLTVDKSTSTVYMELSSLRSEDTAVYYCAR

SEQ ID NO: 55 - protein, 120 aa, synthetic construct
  REGION 1..120: note = RB4-G1-019 VH
QVQLVQSGAEVKKPGASVKVSCKASGYTFTSYWMHWVRQAPGQGLEWMGEINPSNGRTNYNEKFKSRVTLTVDKSTSTVYMELSSLRSEDTAVYYCARDRYDEGNAMDYWGQGTTVTVSS

SEQ ID NO: 56 - protein, 450 aa, synthetic construct
  REGION 1..450: note = RB4-G1-019 heavy chain
QVQLVQSGAEVKKPGASVKVSCKASGYTFTSYWMHWVRQAPGQGLEWMGEINPSNGRTNYNEKFKSRVTLTVDKSTSTVYMELSSLRSEDTAVYYCARDRYDEGNAMDYWGQGTTVTVSSASTKGPSVFPLAPSSKSTSGGTAALGCLVKDYFPEPVTVSWNSGALTSGVHTFPAVLQSSGLYSLSSVVTVPSSSLGTQTYICNVNHKPSNTKVDKKVEPKSCDKTHTCPPCPAPELLGGPSVFLFPPKPKDTLMISRTPEVTCVVVDVSHEDPEVKFNWYVDGVEVHNAKTKPREEQYNSTYRVVSVLTVLHQDWLNGKEYKCKVSNKALPAPIEKTISKAKGQPREPQVYTLPPSRDELTKNQVSLTCLVKGFYPSDIAVEWESNGQPENNYKTTPPVLDSDGSFFLYSKLTVDKSRWQQGNVFSCSVMHEALHNHYTQKSLSLSPGK

SEQ ID NO: 57 - protein, 32 aa, synthetic construct
  REGION 1..32: note = RB4-G1-020 H-FR3
RVTMTRDTSTSTVYMELSSLRSEDTAVYYCAR

SEQ ID NO: 58 - protein, 120 aa, synthetic construct
  REGION 1..120: note = RB4-G1-020 VH
QVQLVQSGAEVKKPGASVKVSCKASGYTFTSYWMHWVRQAPGQGLEWMGEINPSNGRTNYNEKFKSRVTMTRDTSTSTVYMELSSLRSEDTAVYYCARDRYDEGNAMDYWGQGTTVTVSS

SEQ ID NO: 59 - protein, 450 aa, synthetic construct
  REGION 1..450: note = RB4-G1-020 heavy chain
QVQLVQSGAEVKKPGASVKVSCKASGYTFTSYWMHWVRQAPGQGLEWMGEINPSNGRTNYNEKFKSRVTMTRDTSTSTVYMELSSLRSEDTAVYYCARDRYDEGNAMDYWGQGTTVTVSSASTKGPSVFPLAPSSKSTSGGTAALGCLVKDYFPEPVTVSWNSGALTSGVHTFPAVLQSSGLYSLSSVVTVPSSSLGTQTYICNVNHKPSNTKVDKKVEPKSCDKTHTCPPCPAPELLGGPSVFLFPPKPKDTLMISRTPEVTCVVVDVSHEDPEVKFNWYVDGVEVHNAKTKPREEQYNSTYRVVSVLTVLHQDWLNGKEYKCKVSNKALPAPIEKTISKAKGQPREPQVYTLPPSRDELTKNQVSLTCLVKGFYPSDIAVEWESNGQPENNYKTTPPVLDSDGSFFLYSKLTVDKSRWQQGNVFSCSVMHEALHNHYTQKSLSLSPGK

SEQ ID NO: 60 - protein, 32 aa, synthetic construct
  REGION 1..32: note = RB4-G1-022 L-FR3
GVPSRFSGSGSGTDYTFTISSLQPEDIATYYC

SEQ ID NO: 61 - protein, 107 aa, synthetic construct
  REGION 1..107: note = RB4-G1-022 VL
DIQMTQSPSSLSASVGDRVTITCRASQDITNYLNWYQQKPGKAPKLLIYYTSRLHSGVPSRFSGSGSGTDYTFTISSLQPEDIATYYCQQGDTLPRTFGQGTRLEIK

SEQ ID NO: 62 - protein, 214 aa, synthetic construct
  REGION 1..214: note = RB4-G1-022 light chain
DIQMTQSPSSLSASVGDRVTITCRASQDITNYLNWYQQKPGKAPKLLIYYTSRLHSGVPSRFSGSGSGTDYTFTISSLQPEDIATYYCQQGDTLPRTFGQGTRLEIKRTVAAPSVFIFPPSDEQLKSGTASVVCLLNNFYPREAKVQWKVDNALQSGNSQESVTEQDSKDSTYSLSSTLTLSKADYEKHKVYACEVTHQGLSSPVTKSFNRGEC

SEQ ID NO: 63 - protein, 330 aa, synthetic construct [sequence omitted]

SEQ ID NO: 64 - protein, 107 aa, synthetic construct [sequence omitted]

SEQ ID NO: 65 - protein, 451 aa, synthetic construct
  REGION 1..451: note = 128-3: Oncoimmune control antibody, heavy chain
EQSLEESGGDLVTPGASLTLTCKASGIDFSNHYYIYWVRQAPGKGLEWIGCIFSGDSASTYYASWAKGRFTISKSSSPTVTLQMTSLTAADTATYFCARGMSTNDWASDLWGPGTMVTVSSASTKGPSVFPLAPSSKSTSGGTAALGCLVKDYFPEPVTVSWNSGALTSGVHTFPAVLQSSGLYSLSSVVTVPSSSLGTQTYICNVNHKPSNTKVDKKVEPKSCDKTHTCPPCPAPELLGGPSVFLFPPKPKDTLMISRTPEVTCVVVDVSHEDPEVKFNWYVDGVEVHNAKTKPREEQYNSTYRVVSVLTVLHQDWLNGKEYKCKVSNKALPAPIEKTISKAKGQPREPQVYTLPPSRDELTKNQVSLTCLVKGFYPSDIAVEWESNGQPENNYKTTPPVLDSDGSFFLYSKLTVDKSRWQQGNVFSCSVMHEALHNHYTQKSLSLSPGK

SEQ ID NO: 66 - protein, 218 aa, synthetic construct
  REGION 1..218: note = 128-3: Oncoimmune control antibody, light chain
ELVMTQTPASVSAAVGGTVTINCQASESINSIYLAWYQQKPGQRPKLLIYRASTLASGVSSRFKGSASGTGFTLTISDLECADAATYYCQQSYDWGDVENTFGGGTEVEIKRTVAAPSVFIFPPSDEQLKSGTASVVCLLNNFYPREAKVQWKVDNALQSGNSQESVTEQDSKDSTYSLSSTLTLSKADYEKHKVYACEVTHQGLSSPVTKSFNRGEC

SEQ ID NO: 67 - protein, 451 aa, synthetic construct
  REGION 1..451: note = C84: Oncoimmune control antibody, heavy chain
QIQLVQSGPELKKPGETVKISCKASGYTFTNYGMNWVKQAPGKGLKWMGWINTYTGEPTYADDFKGRFAFSLETSASTAYLQINNLKNEDMATYFCASIYYHTSLWYFDVWGAGTTVTVSSASTKGPSVFPLAPSSKSTSGGTAALGCLVKDYFPEPVTVSWNSGALTSGVHTFPAVLQSSGLYSLSSVVTVPSSSLGTQTYICNVNHKPSNTKVDKKVEPKSCDKTHTCPPCPAPELLGGPSVFLFPPKPKDTLMISRTPEVTCVVVDVSHEDPEVKFNWYVDGVEVHNAKTKPREEQYNSTYRVVSVLTVLHQDWLNGKEYKCKVSNKALPAPIEKTISKAKGQPREPQVYTLPPSRDELTKNQVSLTCLVKGFYPSDIAVEWESNGQPENNYKTTPPVLDSDGSFFLYSKLTVDKSRWQQGNVFSCSVMHEALHNHYTQKSLSLSPGK

SEQ ID NO: 68 - protein, 219 aa, synthetic construct
  REGION 1..219: note = C84: Oncoimmune control antibodylight chain
DVLMTQTPLSLPVSLGDQASISCRSSQNIVHSNGNTYLEWYLQKPGQSPKLLIYRVSNRFSGVPVRFSGSGSGTDFTLKISRVEAEDLGVYYCFQGSHVPLTFGAGTKLELKRTVAAPSVFIFPPSDEQLKSGTASVVCLLNNFYPREAKVQWKVDNALQSGNSQESVTEQDSKDSTYSLSSTLTLSKADYEKHKVYACEVTHQGLSSPVTKSFNRGEC

SEQ ID NO: 69 - skipped

SEQ ID NO: 70 - protein, 11 aa, synthetic construct
  REGION 1..11: note = 1A2-7/3A2-18/RB4-G1-018/RB4-G1-019/RB4-G1-020/RB4-G1-022/3G9-1 LCDR1 general formula
  SITE 7: note = misc_feature - Xaa = Ser or Thr
RASQDIXNYLN

SEQ ID NO: 71 - protein, 7 aa, synthetic construct
  REGION 1..7: note = 1A2-7/3A2-18/RB4-G1-018/RB4-G1-019/RB4-G1-020/RB4-G1-022/3G9-1/5E11-2 LCDR2 general formula
  SITE 2: note = misc_feature - Xaa = Ala or Thr
  SITE 4: note = misc_feature - Xaa = Asn or Arg
  SITE 6: note = misc_feature - Xaa = His or Gln
YXSXLXS

SEQ ID NO: 72 - skipped

SEQ ID NO: 73 - protein, 30 aa, synthetic construct
  REGION 1..30: note = 1A2-7/3A2-18/RB4-G1-018/RB4-G1-019/RB4-G1-020/RB4-G1-022/3G9-1/5E11-2 H-FR1 general formula
  SITE 1: note = misc_feature - Xaa = Glu or Gln
  SITE 3: note = misc_feature - Xaa = Lys or Gln
  SITE 5: note = misc_feature - Xaa = Glu, Gln or Val
  SITE 6: note = misc_feature - Xaa = Glu or Gln
  SITE 7: note = misc_feature - Xaa = Pro or Ser
  SITE 9: note = misc_feature - Xaa = Ala or Gly
  SITE 10: note = misc_feature - Xaa = Glu or Gly
  SITE 11: note = misc_feature - Xaa = Leu or Val
  SITE 12: note = misc_feature - Xaa = Lys or Val
  SITE 13: note = misc_feature - Xaa = Lys or Gln
  SITE 16: note = misc_feature - Xaa = Ala or Gly
  SITE 18: note = misc_feature - Xaa = Met or Val
  SITE 20: note = misc_feature - Xaa = Leu or Val
  SITE 23: note = misc_feature - Xaa = Ala or Lys
  SITE 27: note = misc_feature - Xaa = Phe or Tyr
  SITE 30: note = misc_feature - Xaa = Ser or Thr
XVXLXXXGXXXXXPGXSXKXSCXASGXTFX

SEQ ID NO: 74 - protein, 14 aa, synthetic construct
  REGION 1..14: note = 1A2-7/3A2-18/RB4-G1-018/RB4-G1-019/RB4-G1-020/RB4-G1-022/3G9-1/5E11-2 H-FR2 general formula
  SITE 3: note = misc_feature - Xaa = Lys or Arg
  SITE 5: note = misc_feature - Xaa = Ala, Arg or Ser
  SITE 7: note = misc_feature - Xaa = Glu or Gly
  SITE 8: note = misc_feature - Xaa = Lys or Gln
  SITE 13: note = misc_feature - Xaa = Ile, Met or Val
  SITE 14: note = misc_feature - Xaa = Ala or Gly
WVXQXPXXGLEWXX

SEQ ID NO: 75 - protein, 32 aa, synthetic construct
  REGION 1..32: note = 1A2-7/3A2-18/RB4-G1-018/RB4-G1-019/RB4-G1-020/RB4-G1-022/3G9-1/5E11-2 H-FR3 general formula
  SITE 1: note = misc_feature - Xaa = Lys or Arg
  SITE 2: note = misc_feature - Xaa = Ala, Phe or Val
  SITE 4: note = misc_feature - Xaa = Ile, Leu or Met
  SITE 5: note = misc_feature - Xaa = Ile, Ser or Thr
  SITE 6: note = misc_feature - Xaa = Arg or Val
  SITE 8: note = misc_feature - Xaa = Asp, Lys or Thr
  SITE 10: note = misc_feature - Xaa = Lys, Ser or Thr
  SITE 12: note = misc_feature - Xaa = Ser or Thr
  SITE 13: note = misc_feature - Xaa = Ala or Val
  SITE 15: note = misc_feature - Xaa = Leu, Met or Val
  SITE 16: note = misc_feature - Xaa = Glu or Gln
  SITE 17: note = misc_feature - Xaa = Leu or Met
  SITE 18: note = misc_feature - Xaa = Asn or Ser
  SITE 21: note = misc_feature - Xaa = Arg or Thr
  SITE 22: note = misc_feature - Xaa = Ala or Ser
  SITE 25: note = misc_feature - Xaa = Ser or Thr
  SITE 26: note = misc_feature - Xaa = Ala or Gly
  SITE 27: note = misc_feature - Xaa = Ile or Val
  SITE 31: note = misc_feature - Xaa = Ala or Thr
XXTXXXDXSXSXXYXXXXSLXXEDXXXYYCXR

SEQ ID NO: 76 - protein, 11 aa, synthetic construct
  REGION 1..11: note = 1A2-7/3A2-18/RB4-G1-018/RB4-G1-019/RB4-G1-020/RB4-G1-022/3G9-1/5E11-2 H-FR4 general formula
  SITE 6: note = misc_feature - Xaa = Ser or Thr
WGQGTXVTVSS

SEQ ID NO: 77 - protein, 23 aa, synthetic construct
  REGION 1..23: note = 1A2-7/3A2-18/RB4-G1-018/RB4-G1-019/RB4-G1-020/RB4-G1-022/3G9-1/5E11-2 L-FR1 general formula
  SITE 3: note = misc_feature - Xaa = Gln or Val
  SITE 6: note = misc_feature - Xaa = His or Gln
  SITE 7: note = misc_feature - Xaa = Ser or Thr
  SITE 8: note = misc_feature - Xaa = Pro or Thr
  SITE 9: note = misc_feature - Xaa = Ala or Ser
  SITE 12: note = misc_feature - Xaa = Ala or Ser
  SITE 13: note = misc_feature - Xaa = Ala or Val
  SITE 15: note = misc_feature - Xaa = Leu or Val
  SITE 17: note = misc_feature - Xaa = Asp or Gln
  SITE 19: note = misc_feature - Xaa = Ala or Val
  SITE 22: note = misc_feature - Xaa = Ser or Thr
DIXMTXXXXSLXXSXGXRXTIXC

SEQ ID NO: 78 - protein, 15 aa, synthetic construct
  REGION 1..15: note = 1A2-7/3A2-18/RB4-G1-018/RB4-G1-019/RB4-G1-020/RB4-G1-022/3G9-1/5E11-2 L-FR2 general formula
  SITE 7: note = misc_feature - Xaa = Asp or Gly
  SITE 8: note = misc_feature - Xaa = Gly, Lys or Gln
  SITE 9: note = misc_feature - Xaa = Ala, Pro or Thr
  SITE 10: note = misc_feature - Xaa = Pro or Val
  SITE 15: note = misc_feature - Xaa = Lys or Tyr
WYQQKPXXXXKLLIX

SEQ ID NO: 79 - protein, 32 aa, synthetic construct
  REGION 1..32: note = 1A2-7/3A2-18/RB4-G1-018/RB4-G1-019/RB4-G1-020/RB4-G1-022/3G9-1/5E11-2 L-FR3 general formula
  SITE 4: note = misc_feature - Xaa = Ala or Ser
  SITE 14: note = misc_feature - Xaa = Asp or Glu
  SITE 15: note = misc_feature - Xaa = Phe or Tyr
  SITE 16: note = misc_feature - Xaa = Ser or Thr
  SITE 17: note = misc_feature - Xaa = Phe or Leu
  SITE 18: note = misc_feature - Xaa = Asn or Thr
  SITE 20: note = misc_feature - Xaa = His or Ser
  SITE 21: note = misc_feature - Xaa = Asn, Pro or Ser
  SITE 22: note = misc_feature - Xaa = Leu or Val
  SITE 23: note = misc_feature - Xaa = Glu or Gln
  SITE 24: note = misc_feature - Xaa = Glu, Pro or Gln
  SITE 25: note = misc_feature - Xaa = Asp or Glu
  SITE 27: note = misc_feature - Xaa = Phe, Ile or Ser
  SITE 31: note = misc_feature - Xaa = Phe or Tyr
GVPXRFSGSGSGTXXXXXIXXXXXXDXATYXC

SEQ ID NO: 80 - protein, 10 aa, synthetic construct
  REGION 1..10: note = 1A2-7/3A2-18/RB4-G1-018/RB4-G1-019/RB4-G1-020/RB4-G1-022/3G9-1/5E11-2 L-FR4 general formula
  SITE 3: note = misc_feature - Xaa = Gly or Gln
  SITE 6: note = misc_feature - Xaa = Lys or Arg
FGXGTXLEIK

SEQ ID NO: 81 - protein, 120 aa, synthetic construct
  REGION 1..120: note = 1A2-7/3A2-18/RB4-G1-019/RB4-G1-018/RB4-G1-022/RB4-G1-020 VH general formula
  SITE 1: note = misc_feature - Xaa = Glu or Gln
  SITE 5: note = misc_feature - Xaa = Gln or Val
  SITE 7: note = misc_feature - Xaa = Pro or Ser
  SITE 11: note = misc_feature - Xaa = Leu or Val
  SITE 12: note = misc_feature - Xaa = Lys or Val
  SITE 20: note = misc_feature - Xaa = Leu or Val
  SITE 38: note = misc_feature - Xaa = Lys or Arg
  SITE 40: note = misc_feature - Xaa = Ala or Arg
  SITE 48: note = misc_feature - Xaa = Ile or Met
  SITE 67: note = misc_feature - Xaa = Lysor Arg
  SITE 68: note = misc_feature - Xaa = Ala or Val
  SITE 70: note = misc_feature - Xaa = Leu or Met
  SITE 72: note = misc_feature - Xaa = Arg or Val
  SITE 74: note = misc_feature - Xaa = Lys or Thr
  SITE 76: note = misc_feature - Xaa = Ser or Thr
  SITE 79: note = misc_feature - Xaa = Ala or Val
  SITE 81: note = misc_feature - Xaa = Met or Val
  SITE 82: note = misc_feature - Xaa = Glu or Gln
  SITE 84: note = misc_feature - Xaa = Asn or Ser
  SITE 87: note = misc_feature - Xaa = Arg or Thr
  SITE 91: note = misc_feature - Xaa = Ser or Thr
  SITE 115: note = misc_feature - Xaa = Ser or Thr
XVQLXQXGAEXXKPGASVKXSCKASGYTFTSYWMHWVXQXPGQGLEWXGEINPSNGRTNYNEKFKSXXTXTXDXSXSTXYXXLXSLXSEDXAVYYCARDRYDEGNAMDYWGQGTXVTVSS

SEQ ID NO: 82 - protein, 107 aa, synthetic construct
  REGION 1..107: note = 1A2-7/3A2-18/3G9-1/RB4-G1-018/RB4-G1-019/RB4-G1-020/RB4-G1-022 VL general formula
  SITE 3: note = misc_feature - Xaa = Gln or Val
  SITE 6: note = misc_feature - Xaa = His or Gln
  SITE 7: note = misc_feature - Xaa = Ser or Thr
  SITE 8: note = misc_feature - Xaa = Pro or Thr
  SITE 15: note = misc_feature - Xaa = Leu or Val
  SITE 22: note = misc_feature - Xaa = Ser or Thr
  SITE 30: note = misc_feature - Xaa = Ser or Thr
  SITE 41: note = misc_feature - Xaa = Asp or Gly
  SITE 42: note = misc_feature - Xaa = Gly or Lys
  SITE 43: note = misc_feature - Xaa = Ala or Thr
  SITE 44: note = misc_feature - Xaa = Pro or Val
  SITE 70: note = misc_feature - Xaa = Asp or Glu
  SITE 72: note = misc_feature - Xaa = Ser or Thr
  SITE 73: note = misc_feature - Xaa = Phe or Leu
  SITE 77: note = misc_feature - Xaa = Asn or Ser
  SITE 79: note = misc_feature - Xaa = Glu or Gln
  SITE 80: note = misc_feature - Xaa = Pro or Gln
  SITE 81: note = misc_feature - Xaa = Asp or Glu
  SITE 83: note = misc_feature - Xaa = Phe or Ile
  SITE 87: note = misc_feature - Xaa = Phe or Tyr
  SITE 92: note = misc_feature - Xaa = Asp or Asn
  SITE 96: note = misc_feature - Xaa = Pro or Arg
  SITE 100: note = misc_feature - Xaa = Gly or Gln
  SITE 103: note = misc_feature - Xaa = Lys or Arg
DIXMTXXXSSLSASXGDRVTIXCRASQDIXNYLNWYQQKPXXXXKLLIYYTSRLHSGVPSRFSGSGSGTXYXXTISXLXXXDXATYXCQQGXTLPXTFGXGTXLEIK

SEQ ID NO: 83 - protein, 12 aa, synthetic construct
  REGION 1..12: note = 1A2-7/3A2-18/RB4-G1-018/RB4-G1-019/RB4-G1-020/RB4-G1-022/3G9-1 HCDR3 general formula
  SITE 1: note = misc_feature - Xaa = Gly or does not exist
  SITE 2: note = misc_feature - Xaa = Asp or Ile
  SITE 3: note = misc_feature - Xaa = Arg or Tyr
  SITE 5: note = misc_feature - Xaa = Asp or Gly
  SITE 6: note = misc_feature - Xaa = Glu or Tyr
  SITE 7: note = misc_feature - Xaa = Asp or Gly
  SITE 8: note = misc_feature - Xaa = Asn or Tyr
XXXYXXXXAMDY

SEQ ID NO: 84 - protein, 238 aa, synthetic construct
  REGION 1..238: note = human LILRB4 extracellular domain
QAGPLPKPTLWAEPGSVISWGNSVTIWCQGTLEAREYRLDKEESPAPWDRQNPLEPKNKARFSIPSMTEDYAGRYRCYYRSPVGWSQPSDPLELVMTGAYSKPTLSALPSPLVTSGKSVTLLCQSRSPMDTFLLIKERAAHPLLHLRSEHGAQQHQAEFPMSPVTSVHGGTYRCFSSHGFSHYLLSHPSDPLELIVSGSLEDPRPSPTRSVSTAAGPEDQPLMPTGSVPHSGLRRHWE

SEQ ID NO: 85 - protein, 469 aa, synthetic construct
  REGION 1..469: note = LILRB4-Fc
QAGPLPKPTLWAEPGSVISWGNSVTIWCQGTLEAREYRLDKEESPAPWDRQNPLEPKNKARFSIPSMTEDYAGRYRCYYRSPVGWSQPSDPLELVMTGAYSKPTLSALPSPLVTSGKSVTLLCQSRSPMDTFLLIKERAAHPLLHLRSEHGAQQHQAEFPMSPVTSVHGGTYRCFSSHGFSHYLLSHPSDPLELIVSGSLEDPRPSPTRSVSTAAGPEDQPLMPTGSVPHSGLRRHWEPKSCDKTHTCPPCPAPELLGGPSVFLFPPKPKDTLMISRTPEVTCVVVDVSHEDPEVKFNWYVDGVEVHNAKTKPREEQYNSTYRVVSVLTVLHQDWLNGKEYKCKVSNKALPAPIEKTISKAKGQPREPQVYTLPPSREEMTKNQVSLTCLVKGFYPSDIAVEWESNGQPENNYKTTPPVLDSDGSFFLYSKLTVDKSRWQQGNVFSCSVMHEALHNHYTQKSLSLSPGK

SEQ ID NO: 86 - protein, 450 aa, synthetic construct
  REGION 1..450: note = 1A2-7 heavy chain
QVQLQQPGAELVKPGASVKLSCKASGYTFTSYWMHWVKQRPGQGLEWIGEINPSNGRTNYNEKFKSKATLTVDKSSSTAYMQLNSLTSEDSAVYYCARDRYDEGNAMDYWGQGTSVTVSSASTKGPSVFPLAPSSKSTSGGTAALGCLVKDYFPEPVTVSWNSGALTSGVHTFPAVLQSSGLYSLSSVVTVPSSSLGTQTYICNVNHKPSNTKVDKKVEPKSCDKTHTCPPCPAPELLGGPSVFLFPPKPKDTLMISRTPEVTCVVVDVSHEDPEVKFNWYVDGVEVHNAKTKPREEQYNSTYRVVSVLTVLHQDWLNGKEYKCKVSNKALPAPIEKTISKAKGQPREPQVYTLPPSRDELTKNQVSLTCLVKGFYPSDIAVEWESNGQPENNYKTTPPVLDSDGSFFLYSKLTVDKSRWQQGNVFSCSVMHEALHNHYTQKSLSLSPGK

SEQ ID NO: 87 - protein, 214 aa, synthetic construct
  REGION 1..214: note = 1A2-7/3A2-18 light chain
DIVMTQTTSSLSASLGDRVTISCRASQDITNYLNWYQQKPDGTVKLLIYYTSRLHSGVPSRFSGSGSGTDYSLTISNLEQEDIATYFCQQGDTLPRTFGGGTKLEIKRTVAAPSVFIFPPSDEQLKSGTASVVCLLNNFYPREAKVQWKVDNALQSGNSQESVTEQDSKDSTYSLSSTLTLSKADYEKHKVYACEVTHQGLSSPVTKSFNRGEC

SEQ ID NO: 88 - protein, 450 aa, synthetic construct
  REGION 1..450: note = 3A2-18 heavy chain
EVQLQQPGAELVKPGASVKLSCKASGYTFTSYWMHWVKQRPGQGLEWIGEINPSNGRTNYNEKFKSKATLTVDKSSSTAYVQLNSLTSEDSAVYYCARDRYDEGNAMDYWGQGTSVTVSSASTKGPSVFPLAPSSKSTSGGTAALGCLVKDYFPEPVTVSWNSGALTSGVHTFPAVLQSSGLYSLSSVVTVPSSSLGTQTYICNVNHKPSNTKVDKKVEPKSCDKTHTCPPCPAPELLGGPSVFLFPPKPKDTLMISRTPEVTCVVVDVSHEDPEVKFNWYVDGVEVHNAKTKPREEQYNSTYRVVSVLTVLHQDWLNGKEYKCKVSNKALPAPIEKTISKAKGQPREPQVYTLPPSRDELTKNQVSLTCLVKGFYPSDIAVEWESNGQPENNYKTTPPVLDSDGSFFLYSKLTVDKSRWQQGNVFSCSVMHEALHNHYTQKSLSLSPGK

SEQ ID NO: 89 - protein, 451 aa, synthetic construct
  REGION 1..451: note = 3G9-1 heavy chain
QVQLQQPGAELVKPGASVKLSCKASGYTFTSYWMHWVKQRPGQGLEWIGEINPSNGRTNYNEKFKSKATLIVDKSSSTAYMQLSSLTSEDSAVYYCARGIYYGYDYAMDYWGQGTSVTVSSASTKGPSVFPLAPSSKSTSGGTAALGCLVKDYFPEPVTVSWNSGALTSGVHTFPAVLQSSGLYSLSSVVTVPSSSLGTQTYICNVNHKPSNTKVDKKVEPKSCDKTHTCPPCPAPELLGGPSVFLFPPKPKDTLMISRTPEVTCVVVDVSHEDPEVKFNWYVDGVEVHNAKTKPREEQYNSTYRVVSVLTVLHQDWLNGKEYKCKVSNKALPAPIEKTISKAKGQPREPQVYTLPPSRDELTKNQVSLTCLVKGFYPSDIAVEWESNGQPENNYKTTPPVLDSDGSFFLYSKLTVDKSRWQQGNVFSCSVMHEALHNHYTQKSLSLSPGK

SEQ ID NO: 90 - protein, 214 aa, synthetic construct
  REGION 1..214: note = 3G9-1 light chain
DIQMTHTTSSLSASLGDRVTISCRASQDISNYLNWYQQKPDGTVKLLIYYTSRLHSGVPSRFSGSGSGTDYSLTISNLEQEDIATYFCQQGNTLPPTFGGGTKLEIKRTVAAPSVFIFPPSDEQLKSGTASVVCLLNNFYPREAKVQWKVDNALQSGNSQESVTEQDSKDSTYSLSSTLTLSKADYEKHKVYACEVTHQGLSSPVTKSFNRGEC

SEQ ID NO: 91 - protein, 449 aa, synthetic construct
  REGION 1..449: note = 5E11-2 heavy chain
EVKLEESGGGLVQPGGSMKLSCAASGFTFSDAWMDWVRQSPEKGLEWVAEIRSKPNNHATYYAESVKGRFTISRDDSKSSVYLQMNSLRAEDTGIYYCTRTTDYSMDYWGQGTSVTVSSASTKGPSVFPLAPSSKSTSGGTAALGCLVKDYFPEPVTVSWNSGALTSGVHTFPAVLQSSGLYSLSSVVTVPSSSLGTQTYICNVNHKPSNTKVDKKVEPKSCDKTHTCPPCPAPELLGGPSVFLFPPKPKDTLMISRTPEVTCVVVDVSHEDPEVKFNWYVDGVEVHNAKTKPREEQYNSTYRVVSVLTVLHQDWLNGKEYKCKVSNKALPAPIEKTISKAKGQPREPQVYTLPPSRDELTKNQVSLTCLVKGFYPSDIAVEWESNGQPENNYKTTPPVLDSDGSFFLYSKLTVDKSRWQQGNVFSCSVMHEALHNHYTQKSLSLSPGK

SEQ ID NO: 92 - protein, 218 aa, synthetic construct
  REGION 1..218: note = 5E11-2 light chain
DIQMTQSPASLAVSLGQRATISCRASQSVSASSYSYMHWYQQKPGQPPKLLIKYASNLQSGVPARFSGSGSGTDFTLNIHPVEEEDSATYYCQHSWEIPRTFGGGTKLEIKRTVAAPSVFIFPPSDEQLKSGTASVVCLLNNFYPREAKVQWKVDNALQSGNSQESVTEQDSKDSTYSLSSTLTLSKADYEKHKVYACEVTHQGLSSPVTKSFNRGEC